European Patent Specification EP 4 089 106 B1, published April 16, 2025. Title: A new anti-metabolic disorder FGF analog and its application. Applicant: Jiangnan University. The sequence listing filed with the application follows.

SEQUENCE LISTING (8 sequences)

SEQ ID NO: 1 - protein, 189 aa, Artificial Sequence
  Protein translated from synthetic DNA
MRDSSPLVHYGWGDPIRLRHLYTSGPHGLSSCFLRIRADGVVDCARGQSAHSLLEIKAVALRTVAIKGVHSVRYLCMGADGKMQGLLQYSEEDCAFEEEIRPDGYNVYRSEKHRLPVCLSSAKQRQLYKNRGFLPLCHFLPMLPMVPEEPEDLRGHLESDMFSSPPDVGSSDPLSMVGPSQGRSPSYAS

SEQ ID NO: 2 - protein, 178 aa, Artificial Sequence
  Protein translated from synthetic DNA
MRDSSPLVHYGWGDPIRLRHLYTSGPHGLSSCFLRIRADGVVDCARGQSAHSLLEIKAVALRTVAIKGVHSVRYLCMGADGKMQGLLQYSEEDCAFEEEIRPDGYNVYRSEKHRLPVCLSSAKQRQLYKNRGFLPLPGLPPALPEPPGILAPQPPDVGSSDPLSMVGPSQGRSPSYAS

SEQ ID NO: 3 - protein, 191 aa, Artificial Sequence
  Protein translated from synthetic DNA
MADSSPLLQFGGQVRQRYLYTDDAQRTEAHLEIREDGTVGGAADQSPESLLQLKALKPGVIQILGVRTPRFLCQRPDGALYGSLHFDPEACSFRELLLEDGYNVYQSEAHGLPLHLPGNKSPHRDPAPRGPARFLPLCHFLPMLPMVPEEPEDLRGHLESDMFSSPLETDSMDPFGLVTGLEAVRSPSFEK

SEQ ID NO: 4 - protein, 180 aa, Artificial Sequence
  Protein translated from synthetic DNA
MADSSPLLQFGGQVRQRYLYTDDAQRTEAHLEIREDGTVGGAADQSPESLLQLKALKPGVIQILGVRTPRFLCQRPDGALYGSLHFDPEACSFRELLLEDGYNVYQSEAHGLPLHLPGNKSPHRDPAPRGPARFLPLPGLPPALPEPPGILAPQPLETDSMDPFGLVTGLEAVRSPSFEK

SEQ ID NO: 5 - DNA, 567 bp, Artificial Sequence
  Synthetic DNA
atgcgtgatagcagcccgctggttcattatggttggggtgatccgattcgtctgcgtcatctgtataccagcggtccgcatggtctgagcagctgttttctgcgtattcgtgcagatggtgttgttgattgtgcacgtggtcagagcgcacatagcctgctggaaattaaagcagttgcactgcgtaccgttgcaattaaaggtgttcatagcgttcgttatctgtgtatgggtgcagatggtaaaatgcagggtctgctgcagtatagcgaagaagattgtgcatttgaagaagaaattcgtccggatggttataatgtttatcgtagcgaaaaacatcgtctgccggtttgcctgagcagcgcaaaacagcgtcagctgtataaaaatcgtggttttctgccgctgtgccattttctgccgatgctgccgatggttccggaagaaccggaagatctgcgtggtcatctggaaagcgatatgtttagcagcccgcccgatgtgggctcctcggaccctctgagcatggtgggaccttcccagggccgaagccccagctacgcttcc

SEQ ID NO: 6 - DNA, 537 bp, Artificial Sequence
  Synthetic DNA
atgcgtgatagcagcccgctggttcattatggttggggtgatccgattcgtctgcgtcatctgtataccagcggtccgcatggtctgagcagctgttttctgcgtattcgtgcagatggtgttgttgattgtgcacgtggtcagagcgcacatagcctgctggaaattaaagcagttgcactgcgtaccgttgcaattaaaggtgttcatagcgttcgttatctgtgtatgggtgcagatggtaaaatgcagggtctgctgcagtatagcgaagaagattgtgcatttgaagaagaaattcgtccggatggttataatgtttatcgtagcgaaaaacatcgtctgccggtttgcctgagcagcgcaaaacagcgtcagctgtataaaaatcgtggttttctgccgctgccaggcctgccccccgcactcccggagccacccggaatcctggccccccagccccccgatgtgggctcctcggaccctctgagcatggtgggaccttcccagggccgaagccccagctacgcttcctga

SEQ ID NO: 7 - DNA, 576 bp, Artificial Sequence
  Synthetic DNA
atggcagactccagtcctctcctgcaattcgggggccaagtccggcagcggtacctctacacagatgatgcccagcgtacagaagcccacctggagatcagggaggatgggacggtggggggcgctgctgaccagagccccgaaagtctcctgcagctgaaagccttgaagccgggagttattcaaatcttgggagtccgtacaccgaggttcctgtgccagcggccagatggggccctgtatggatcgctccactttgaccctgaggcctgcagcttccgggagctgcttcttgaggacggatacaatgtttaccagtccgaagcccacggcctcccgctgcacctgccagggaacaagtccccacaccgggaccctgcaccccgaggaccagctcgcttcctgccactatgccattttctgccgatgctgccgatggttccggaagaaccggaagatctgcgtggtcatctggaaagcgatatgtttagcagcccgctggaaaccgatagcatggacccgtttggtctggttaccggtctggaagcagttcgtagcccgagctttgaaaaataa

SEQ ID NO: 8 - DNA, 543 bp, Artificial Sequence
  Synthetic DNA
atggcagactccagtcctctcctgcaattcgggggccaagtccggcagcggtacctctacacagatgatgcccagcgtacagaagcccacctggagatcagggaggatgggacggtggggggcgctgctgaccagagccccgaaagtctcctgcagctgaaagccttgaagccgggagttattcaaatcttgggagtccgtacaccgaggttcctgtgccagcggccagatggggccctgtatggatcgctccactttgaccctgaggcctgcagcttccgggagctgcttcttgaggacggatacaatgtttaccagtccgaagcccacggcctcccgctgcacctgccagggaacaagtccccacaccgggaccctgcaccccgaggaccagctcgcttcctgccactaccaggcctgccccccgcactcccggagccacccggaatcctggccccccagcccctggaaaccgatagcatggacccgtttggtctggttaccggtctggaagcagttcgtagcccgagctttgaaaaataa